European Patent Application EP 4 434 523 A1, published September 25, 2024. Title: Agent for treatment of neutropenia. Applicant: Eberhard Karls Universität Tübingen - Medizinische Fakultät. The sequence listing filed with the application follows.

SEQUENCE LISTING (12 sequences)

SEQ ID NO: 1 - DNA, 20 bp, synthetic construct
  source 1..20: mol_type = other DNA
ctgcgcggaggccacttctg

SEQ ID NO: 2 - DNA, 20 bp, synthetic construct
  source 1..20: mol_type = other DNA
gggacgccgcctgggcaacg

SEQ ID NO: 3 - DNA, 20 bp, synthetic construct
  source 1..20: mol_type = other DNA
ttagcccgttgcagaccaag

SEQ ID NO: 4 - DNA, 123 bp, synthetic construct
  source 1..123: mol_type = other DNA
cggccccacgcgtggcccttcatggtgtccctgcagctgcgcggaggccacttctgcggcgccaccctgattgcgcccaacttcgtcatgtcggccgcgcactgcgtggcgaatgtgtgagta

SEQ ID NO: 5 - DNA, 123 bp, synthetic construct
  source 1..123: mol_type = other DNA
gccaacgtgcaggtggcccagctgccggctcagggacgccgcctgggcaacggggtgcagtgcctggccatgggctggggccttctgggcaggaaccgtgggatcgccagcgtcctgcaggag

SEQ ID NO: 6 - DNA, 123 bp, synthetic construct
  source 1..123: mol_type = other DNA
cggggcaaaggcatcggggtagagccctgaggcgcagcctccccggacgaaggaggcaattccgtggattagcccgttgcagaccaaggggctgccggagtccccctgtggaggcagacaagg

SEQ ID NO: 7 - DNA, 20 bp, synthetic construct
  source 1..20: mol_type = other DNA
ggctccttggcaggcactca

SEQ ID NO: 8 - DNA, 20 bp, synthetic construct
  source 1..20: mol_type = other DNA
cacctcacagaccgggacgc

SEQ ID NO: 9 - DNA, 20 bp, synthetic construct
  source 1..20: mol_type = other DNA
cgccctgagccttggtgacg

SEQ ID NO: 10 - DNA, 20 bp, synthetic construct
  source 1..20: mol_type = other DNA
agccacggtgcctgttgctg

SEQ ID NO: 11 - DNA, 20 bp, synthetic construct
  source 1..20: mol_type = other DNA
cagcccggactgcagcaaca

SEQ ID NO: 12 - DNA, 20 bp, synthetic construct
  source 1..20: mol_type = other DNA
gacccgggcagcccttctca